European Patent Application EP 4 299 124 A1, published January 3, 2024. Title: Anti-mGluR2 nanobodies for use as biomolecule transporter. Applicant: Université de Montpellier Centre National de la Recherche Scientifique (CNRS) INSERM (Institut National de la Santé et de la Recherche Médicale). The sequence listing filed with the application follows.

SEQUENCE LISTING (53 sequences)

SEQ ID NO: 1 - protein, 8 aa, artificial
  CDR1 sequence of IGF-1159 nanobody
GRTFSSFA

SEQ ID NO: 2 - protein, 7 aa, artificial
  CDR2 sequence of IGF-1159 nanobody
ISWSGST

SEQ ID NO: 3 - protein, 17 aa, artificial
  CDR3 sequence of IGF-1159 nanobody
ALGKGSSYYYSPSGYDY

SEQ ID NO: 4 - protein, 8 aa, artificial
  CDR1 sequence of IGF-1160 nanobody
GRTFSTYG

SEQ ID NO: 5 - protein, 8 aa, artificial
  CDR2 sequence of IGF-1160 nanobody
INWRDDVT

SEQ ID NO: 6 - protein, 19 aa, artificial
  CDR3 sequence of IGF-1160 nanobody
AAQGRGSFKSIFERSRYDS

SEQ ID NO: 7 - protein, 8 aa, artificial
  CDR1 sequence of IGF-1164 nanobody
GRTFSDLA

SEQ ID NO: 8 - protein, 8 aa, artificial
  CDR2 sequence of IGF-1164 nanobody
INWSGHSI

SEQ ID NO: 9 - protein, 18 aa, artificial
  CDR3 sequence of IGF-1164 nanobody
AADTTGGTYKLRTKEYDY

SEQ ID NO: 10 - protein, 8 aa, artificial
  CDR1 sequence of IGF-1163 nanobody
GRTFRPYG

SEQ ID NO: 11 - protein, 8 aa, artificial
  CDR2 sequence of IGF-1163 nanobody
IIWSLGYT

SEQ ID NO: 12 - protein, 12 aa, artificial
  CDR3 sequence of IGF-1163 nanobody
AARDRSSSEYDY

SEQ ID NO: 13 - protein, 8 aa, artificial
  CDR1 sequence of IGF-1166 nanobody
GRTFSIYS

SEQ ID NO: 14 - protein, 8 aa, artificial
  CDR2 sequence of IGF-1166 nanobody
ITWRREYT

SEQ ID NO: 15 - protein, 12 aa, artificial
  CDR3 sequence of IGF-1166 nanobody
ALRPGLRDDLNY

SEQ ID NO: 16 - protein, 8 aa, artificial
  CDR1 sequence of IGF-1168 nanobody
VRFFSINT

SEQ ID NO: 17 - protein, 7 aa, artificial
  CDR2 sequence of IGF-1168 nanobody
ITSSGST

SEQ ID NO: 18 - protein, 12 aa, artificial
  CDR3 sequence of IGF-1168 nanobody
HADYKYTTHNTA

SEQ ID NO: 19 - protein, 123 aa, artificial
  amino acid sequence of IGF-1159 nanobody
QVQLVQSGGGLVQAGGSLRLSCAASGRTFSSFAMAWFRQAPGKEREFVAAISWSGSTGHADSVKGRFTITRDNAKNTVFLQMNSLKPEDTAVYYCALGKGSSYYYSPSGYDYWGQGTQVTVSS

SEQ ID NO: 20 - protein, 126 aa, artificial
  amino acid sequence of IGF-1160 nanobody
EVQLVESGGGLVQAGDSLRLSCAASGRTFSTYGMAWFRQAPGKEREFVARINWRDDVTYYADSLKGRFTISRDKAKNTVYLQLDSLTPEDTAVYYCAAQGRGSFKSIFERSRYDSWGQGTQVTVSS

SEQ ID NO: 21 - protein, 125 aa, artificial
  amino acid sequence of IGF-1164 nanobody
EVQLVESGGGLVQAGGSLRLSCAASGRTFSDLAMGWFRQAPGKEREFVAAINWSGHSIYYTDSVKARFTISRDNAKDTVYLQMNSLKSEDTAVYFCAADTTGGTYKLRTKEYDYRGQGTQVTVSS

SEQ ID NO: 22 - protein, 119 aa, artificial
  amino acid sequence of IGF-1163nanobody
QVQLVQSGGGYVQAGGSLSVSCAASGRTFRPYGVGWFRQAPGKEREFVAAIIWSLGYTIYADSVKGRFTISRDNAKNTVYLQMNSLKAEDTAVYYCAARDRSSSEYDYWGQGTQVTVSS

SEQ ID NO: 23 - protein, 119 aa, artificial
  amino acid sequence of IGF-1166 nanobody
EVQLVESGGGVVQPGDSLRLSCVASGRTDSIYSMAWFRQAPGKEREFVAIITWRREYTNYEDSVRGRFTISRDNAKNAVYLQMNKLKPEDTAVYYCALRPGLRDDLNYWGQGTQVTVSS

SEQ ID NO: 24 - protein, 118 aa, artificial
  amino acid sequence of IGF-1168 nanobody
QVQLVQSGGGLVQAGGSLRLSCAASVRFFSINTMGWYRQAPGKQRELVADITSSGSTNYADSGKGRFTISRDNAKNTVYLQMNRLKPEDTAVYYCHADYKYTTHNTAWGQGTQVTVSS

SEQ ID NO: 25 - protein, 29 aa, artificial
  linker sequence L1
EPKIPQPQPKPQPQPQPQPQPKPQPKPEP

SEQ ID NO: 26 - protein, 15 aa, artificial
  linker sequence L2
GGGGSGGGGSGGGGS

SEQ ID NO: 27 - protein, 20 aa, artificial
  linker sequence L3
GGGGSGGGGSGGGGSGGGGS

SEQ ID NO: 28 - protein, 5 aa, artificial
  linker sequence L4
GGGGS

SEQ ID NO: 29 - protein, 3 aa, artificial
  linker sequence L5
GGS

SEQ ID NO: 30 - protein, 3 aa, artificial
  linker sequence L6
GGG

SEQ ID NO: 31 - protein, 15 aa, artificial
  linker sequence L7
GGGSSGGGSSGGGSS

SEQ ID NO: 32 - protein, 270 aa, artificial
  Amino acid sequence of the biparatopic IGF1202 (construct IGF1168-linker sequenceL1-IGF1159)
QVQLVQSGGGLVQAGGSLRLSCAASVRFFSINTMGWYRQAPGKQRELVADITSSGSTNYADSGKGRFTISRDNAKNTVYLQMNRLKPEDTAVYYCHADYKYTTHNTAWGQGTQVTVSSEPKIPQPQPKPQPQPQPQPQPKPQPKPEPQVQLVQSGGGLVQAGGSLRLSCAASGRTFSSFAMAWFRQAPGKEREFVAAISWSGSTGHADSVKGRFTITRDNAKNTVFLQMNSLKPEDTAVYYCALGKGSSYYYSPSGYDYWGQGTQVTVSS

SEQ ID NO: 33 - protein, 278 aa, artificial
  Amino acid sequence of the biparatopic IGF1202-tag6xHIS
QVQLVQSGGGLVQAGGSLRLSCAASVRFFSINTMGWYRQAPGKQRELVADITSSGSTNYADSGKGRFTISRDNAKNTVYLQMNRLKPEDTAVYYCHADYKYTTHNTAWGQGTQVTVSSEPKIPQPQPKPQPQPQPQPQPKPQPKPEPQVQLVQSGGGLVQAGGSLRLSCAASGRTFSSFAMAWFRQAPGKEREFVAAISWSGSTGHADSVKGRFTITRDNAKNTVFLQMNSLKPEDTAVYYCALGKGSSYYYSPSGYDYWGQGTQVTVSSLEHHHHHH

SEQ ID NO: 34 - DNA, 369 bp, artificial
  nucleic acid sequence of IGF-1159 nanobody
caggtgcagctggtgcagtctgggggaggattggtgcaggctgggggctctctgagactctcctgtgcagcctctggacgcacctttagtagcttcgccatggcctggttccgccaggctccagggaaggagcgtgagtttgtagcagctattagctggagtggtagtacaggccatgcagactctgtgaagggccgattcaccatcaccagagacaacgccaagaacacggtgtttctgcaaatgaacagcctgaaacctgaggacacggccgtttattactgtgcactaggaaaggggagtagttactactacagtcctagtgggtatgactactggggccaggggacccaggtcaccgtctcctca

SEQ ID NO: 35 - DNA, 378 bp, artificial
  nucleic acid sequence of IGF-1160 nanobody
gaggtgcagctggtggagtctggtggaggattggtgcaggctggggactctctgagactctcctgtgcagcctctggacgcacctttagtacctatggcatggcctggttccgccaggctccggggaaggagcgtgagtttgtggcgcgaattaactggcgcgatgatgtcacatactatgcagactccctgaagggccgattcaccatctcccgagacaaagccaagaacacggtgtatctgcaactggacagcctgactcctgaggacacggccgtttattactgtgcagcccaaggtcgcggtagttttaaatcaatcttcgagcggtcgcgctatgactcctggggccaggggacccaggtcaccgtctcctca

SEQ ID NO: 36 - DNA, 375 bp, artificial
  nucleic acid sequence of IGF-1164 nanobody
gaggtgcagctggtggagtctgggggaggattggtgcaggctgggggctctctgagactgtcctgtgcagcctctggacgcaccttcagtgaccttgccatgggctggttccgccaggctccaggaaaggagcgtgagtttgtagcagccattaactggagtggtcatagcatatactatacagactccgtgaaggcccgattcaccatctccagagacaacgccaaagacacggtgtatctgcaaatgaacagcctgaaatctgaggacacggccgtttatttttgtgcagcagatacgactggtggcacctataaactccggacgaaggagtatgactaccgggggcaggggacccaggtcaccgtctcctca

SEQ ID NO: 37 - DNA, 357 bp, artificial
  nucleic acid sequence of IGF-1163 nanobody
caggtgcagctggtgcagtctgggggaggatatgtgcaggctgggggctctctgagcgtctcctgtgcagcctctggacgaaccttccgtccctatggcgtgggctggttccgccaggctccagggaaggagcgtgagtttgtagcagctattatttggagtcttggatacacaatttatgcagactccgtgaagggccgattcaccatctccagagacaacgccaagaacacggtttatctgcaaatgaacagcctgaaagctgaggacacggccgtttattactgtgcagcccgcgatcgtagttcgtcagagtatgactactggggccaggggacccaggtcaccgtctcctca

SEQ ID NO: 38 - DNA, 357 bp, artificial
  nucleic acid sequence of IGF-1166 nanobody
gaggtgcagctggtggagtctgggggaggagtggtgcagcctggggattctctgagactctcttgtgtagcctctggacgcaccgatagtatttattccatggcctggttccgccaggctccagggaaggaacgtgagtttgtagcgattattacctggagacgtgagtacacaaattatgaggactccgtgaggggccgattcaccatctccagagacaacgccaagaacgcggtgtatctgcaaatgaacaagttgaaacctgaggacacggccgtttattactgtgcacttaggccaggcctacgcgatgacttaaactactggggccaggggacccaggtcaccgtctcctca

SEQ ID NO: 39 - DNA, 354 bp, artificial
  nucleic acid sequence of IGF-1168 nanobody
caggtgcagctggtgcagtctgggggaggcttggtgcaggctggggggtctctgagactctcctgtgcagcctctgtaaggttcttcagtattaataccatgggctggtaccgccaggctccagggaagcagcgcgagttggtcgcagatattactagtagtggtagcacaaactatgcagactccgggaagggccgattcaccatctccagagacaacgccaagaacacggtgtatctgcagatgaacaggttgaaacctgaggacacagccgtctattactgccatgcggattacaaatacacaacccataacacggcctggggccaggggacccaggtcaccgtctcctca

SEQ ID NO: 40 - DNA, 810 bp, artificial
  nucleic acid sequence of the biparatopic IGF1202 (construct IGF1168-linker sequenceL1-IGF1159)
caggtgcagcttgtacagtctgggggaggcttggtgcaggctggggggtctctgagactctcctgtgcagcctctgtaaggttcttcagtattaataccatgggctggtatcgccaggctccagggaagcagcgcgagttggtcgcagatattactagtagtggtagcacaaactatgcagactccgggaagggccgattcaccatctccagagacaacgccaagaacacggtgtatctgcagatgaacaggttgaaacctgaggacacagccgtctattactgccatgcggattacaaatacacaacccataacacggcctggggccagggtacccaggtcaccgtctcctcagaaccgaagatcccgcagccgcagccaaaacctcagccgcagccacagccgcaacctcaaccgaaaccgcaaccaaaaccggaacctcaggtgcaattggtgcagtctgggggaggattggtgcaggctgggggctctctgagactctcctgtgcagcctctggacgcacctttagtagcttcgccatggcctggttccgccaggctccagggaaggagcgtgagtttgtagcagctattagctggagtggtagtacaggccatgcagactctgtgaagggccgattcaccatcaccagagacaacgccaagaacacggtgtttctgcaaatgaacagcctgaaacctgaggacacggccgtttattactgtgcactaggaaaggggagtagttactactacagtcctagtgggtatgactactggggccaggggacccaggtcaccgtctcctca

SEQ ID NO: 41 - DNA, 834 bp, artificial
  nucleic acid sequence of the biparatopic IGF1202-tag6xHIS
caggtgcagcttgtacagtctgggggaggcttggtgcaggctggggggtctctgagactctcctgtgcagcctctgtaaggttcttcagtattaataccatgggctggtatcgccaggctccagggaagcagcgcgagttggtcgcagatattactagtagtggtagcacaaactatgcagactccgggaagggccgattcaccatctccagagacaacgccaagaacacggtgtatctgcagatgaacaggttgaaacctgaggacacagccgtctattactgccatgcggattacaaatacacaacccataacacggcctggggccagggtacccaggtcaccgtctcctcagaaccgaagatcccgcagccgcagccaaaacctcagccgcagccacagccgcaacctcaaccgaaaccgcaaccaaaaccggaacctcaggtgcaattggtgcagtctgggggaggattggtgcaggctgggggctctctgagactctcctgtgcagcctctggacgcacctttagtagcttcgccatggcctggttccgccaggctccagggaaggagcgtgagtttgtagcagctattagctggagtggtagtacaggccatgcagactctgtgaagggccgattcaccatcaccagagacaacgccaagaacacggtgtttctgcaaatgaacagcctgaaacctgaggacacggccgtttattactgtgcactaggaaaggggagtagttactactacagtcctagtgggtatgactactggggccaggggacccaggtcaccgtctcctcactcgagcaccaccaccaccaccac

SEQ ID NO: 42 - protein, 115 aa, artificial
  Amino acid sequence of the nanobody against Albumine (Alb8)
QVQLQESGGGLVQPGGSLRLSCEASGFTFSRFGMTWVRQAPGKGVEWVSGISSLGDSTLYADSVKGRFTISRDNAKNTLYLQMNSLKPEDTAVYYCTIGGSLNPGGQGTQVTVSS

SEQ ID NO: 43 - protein, 125 aa, artificial
  Amino acid sequence of the nanobody against Transferin receptor (Tfr)
EVQLQASGGGLVQAGGSLRLSCSASVRTFSIYAMGWFRQAPGKEREFVAGINRSGDVTKYADFVKGRFSISRDNAKNMVYLQMNSLKPEDTALYYCAATWAYDTVGALTSGYNFWGQGTQVTVSS

SEQ ID NO: 44 - protein, 391 aa, artificial
  Amino acid sequence of the biparatopic nanobody IGF-1267 (biparatopic IGF1201 with nanobody against Tfr)
QVQLVQSGGGLVQAGGSLRLSCAASVRFFSINTMGWYRQAPGKQRELVADITSSGSTNYADSGKGRFTISRDNAKNTVYLQMNRLKPEDTAVYYCHADYKYTTHNTAWGQGTQVTVSSGGGGSGGGGSGGGGSQVQLVQSGGGLVQAGGSLRLSCAASGRTFSSFAMAWFRQAPGKEREFVAAISWSGSTGHADSVKGRFTITRDNAKNTVFLQMNSLKPEDTAVYYCALGKGSSYYYSPSGYDYWGQGTQVTVSSGGGGSGGGGSEVQLQASGGGLVQAGGSLRLSCSASVRTFSIYAMGWFRQAPGKEREFVAGINRSGDVTKYADFVKGRFSISRDNAKNMVYLQMNSLKPEDTALYYCAATWAYDTVGALTSGYNFWGQGTQVTVSS

SEQ ID NO: 45 - protein, 405 aa, artificial
  Amino acid sequence of the biparatopic nanobody IGF-1268 (biparatopic IGF1202 with nanobody against Tfr)
QVQLVQSGGGLVQAGGSLRLSCAASVRFFSINTMGWYRQAPGKQRELVADITSSGSTNYADSGKGRFTISRDNAKNTVYLQMNRLKPEDTAVYYCHADYKYTTHNTAWGQGTQVTVSSEPKIPQPQPKPQPQPQPQPQPKPQPKPEPQVQLVQSGGGLVQAGGSLRLSCAASGRTFSSFAMAWFRQAPGKEREFVAAISWSGSTGHADSVKGRFTITRDNAKNTVFLQMNSLKPEDTAVYYCALGKGSSYYYSPSGYDYWGQGTQVTVSSGGGGSGGGGSEVQLQASGGGLVQAGGSLRLSCSASVRTFSIYAMGWFRQAPGKEREFVAGINRSGDVTKYADFVKGRFSISRDNAKNMVYLQMNSLKPEDTALYYCAATWAYDTVGALTSGYNFWGQGTQVTVSS

SEQ ID NO: 46 - protein, 381 aa, artificial
  Amino acid sequence of the biparatopic nanobody IGF-1269 (biparatopic IGF1201 with nanobody against Alb8)
QVQLVQSGGGLVQAGGSLRLSCAASVRFFSINTMGWYRQAPGKQRELVADITSSGSTNYADSGKGRFTISRDNAKNTVYLQMNRLKPEDTAVYYCHADYKYTTHNTAWGQGTQVTVSSGGGGSGGGGSGGGGSQVQLVQSGGGLVQAGGSLRLSCAASGRTFSSFAMAWFRQAPGKEREFVAAISWSGSTGHADSVKGRFTITRDNAKNTVFLQMNSLKPEDTAVYYCALGKGSSYYYSPSGYDYWGQGTQVTVSSGGGGSGGGGSQVQLQESGGGLVQPGGSLRLSCEASGFTFSRFGMTWVRQAPGKGVEWVSGISSLGDSTLYADSVKGRFTISRDNAKNTLYLQMNSLKPEDTAVYYCTIGGSLNPGGQGTQVTVSS

SEQ ID NO: 47 - protein, 395 aa, artificial
  Amino acid sequence of the biparatopic nanobody IGF-1270 (biparatopic IGF1202 with nanobody against Alb8)
QVQLVQSGGGLVQAGGSLRLSCAASVRFFSINTMGWYRQAPGKQRELVADITSSGSTNYADSGKGRFTISRDNAKNTVYLQMNRLKPEDTAVYYCHADYKYTTHNTAWGQGTQVTVSSEPKIPQPQPKPQPQPQPQPQPKPQPKPEPQVQLVQSGGGLVQAGGSLRLSCAASGRTFSSFAMAWFRQAPGKEREFVAAISWSGSTGHADSVKGRFTITRDNAKNTVFLQMNSLKPEDTAVYYCALGKGSSYYYSPSGYDYWGQGTQVTVSSGGGGSGGGGSQVQLQESGGGLVQPGGSLRLSCEASGFTFSRFGMTWVRQAPGKGVEWVSGISSLGDSTLYADSVKGRFTISRDNAKNTLYLQMNSLKPEDTAVYYCTIGGSLNPGGQGTQVTVSS

SEQ ID NO: 48 - DNA, 345 bp, artificial
  Nucleic acid sequence of the nanobody against Albumine (Alb8)
caggtgcagctgcaagaaagcggagggggcctggtccagccaggaggcagcctccggctaagttgcgaggccagcggcttcacattcagtagatttggcatgacatgggtcaggcaggccccaggtaaaggcgtggaatgggtaagcggcataagcagtctgggagacagcacactctacgccgattccgtgaaaggccgcttcaccatctctagagacaacgcaaaaaataccctgtaccttcagatgaattcactcaagcccgaagacacggccgtttattactgcacaatcggcgggtcactaaacccaggcggacaggggacacaagtaacggttagtagc

SEQ ID NO: 49 - DNA, 375 bp, artificial
  Nucleic acid sequence of the nanobody against Transferin receptor (Tfr)
gaagtgcagcttcaggctagcgggggaggcttggtgcaggctggggggtctctgagactctcctgtagcgcctctgtgcggacctttagcatctacgcaatgggctggttccgccaggctccagggaaggaacgcgagttcgtcgcgggcatcaacagaagtggtgacgtaacaaaatacgccgatttcgtaaaggggcgattcagcatctccagagacaacgccaagaacatggtgtatctgcagatgaacagcttgaaacctgaggacacagccctgtattactgcgccgcgacctgggcgtacgacaccgtgggcgcgctgaccagcggctataatttttggggccaaggcacccaggtcaccgtgagctca

SEQ ID NO: 50 - DNA, 1173 bp, artificial
  Nucleic acid sequence of the biparatopic nanobody IGF-1267
caggtgcagcttgtacagtctgggggaggcttggtgcaggctggggggtctctgagactctcctgtgcagcctctgtaaggttcttcagtattaataccatgggctggtatcgccaggctccagggaagcagcgcgagttggtcgcagatattactagtagtggtagcacaaactatgcagactccgggaagggccgattcaccatctccagagacaacgccaagaacacggtgtatctgcagatgaacaggttgaaacctgaggacacagccgtctattactgccatgcggattacaaatacacaacccataacacggcctggggccagggtacccaggtcaccgtctcctcaggtgggggtggcagcggtggcggcggtagcgggggcggtggcagccaggtgcaattggtgcagtctgggggaggattggtgcaggctgggggctctctgagactctcctgtgcagcctctggacgcacctttagtagcttcgccatggcctggttccgccaggctccagggaaggagcgtgagtttgtagcagctattagctggagtggtagtacaggccatgcagactctgtgaagggccgattcaccatcaccagagacaacgccaagaacacggtgtttctgcaaatgaacagcctgaaacctgaggacacggccgtttattactgtgcactaggaaaggggagtagttactactacagtcctagtgggtatgactactggggccaggggacccaggtcaccgtctcctcaggtgggggtggcagcggtggcggcggtagcgaagtgcagcttcaggctagcgggggaggcttggtgcaggctggggggtctctgagactctcctgtagcgcctctgtgcggacctttagcatctacgcaatgggctggttccgccaggctccagggaaggaacgcgagttcgtcgcgggcatcaacagaagtggtgacgtaacaaaatacgccgatttcgtaaaggggcgattcagcatctccagagacaacgccaagaacatggtgtatctgcagatgaacagcttgaaacctgaggacacagccctgtattactgcgccgcgacctgggcgtacgacaccgtgggcgcgctgaccagcggctataatttttggggccaaggcacccaggtcaccgtgagctca

SEQ ID NO: 51 - DNA, 1215 bp, artificial
  Nucleic acid sequence of the biparatopic nanobody IGF-1268
caggtgcagcttgtacagtctgggggaggcttggtgcaggctggggggtctctgagactctcctgtgcagcctctgtaaggttcttcagtattaataccatgggctggtatcgccaggctccagggaagcagcgcgagttggtcgcagatattactagtagtggtagcacaaactatgcagactccgggaagggccgattcaccatctccagagacaacgccaagaacacggtgtatctgcagatgaacaggttgaaacctgaggacacagccgtctattactgccatgcggattacaaatacacaacccataacacggcctggggccagggtacccaggtcaccgtctcctcagaaccgaagatcccgcagccgcagccaaaacctcagccgcagccacagccgcaacctcaaccgaaaccgcaaccaaaaccggaacctcaggtgcaattggtgcagtctgggggaggattggtgcaggctgggggctctctgagactctcctgtgcagcctctggacgcacctttagtagcttcgccatggcctggttccgccaggctccagggaaggagcgtgagtttgtagcagctattagctggagtggtagtacaggccatgcagactctgtgaagggccgattcaccatcaccagagacaacgccaagaacacggtgtttctgcaaatgaacagcctgaaacctgaggacacggccgtttattactgtgcactaggaaaggggagtagttactactacagtcctagtgggtatgactactggggccaggggacccaggtcaccgtctcctcaggtgggggtggcagcggtggcggcggtagcgaagtgcagcttcaggctagcgggggaggcttggtgcaggctggggggtctctgagactctcctgtagcgcctctgtgcggacctttagcatctacgcaatgggctggttccgccaggctccagggaaggaacgcgagttcgtcgcgggcatcaacagaagtggtgacgtaacaaaatacgccgatttcgtaaaggggcgattcagcatctccagagacaacgccaagaacatggtgtatctgcagatgaacagcttgaaacctgaggacacagccctgtattactgcgccgcgacctgggcgtacgacaccgtgggcgcgctgaccagcggctataatttttggggccaaggcacccaggtcaccgtgagctca

SEQ ID NO: 52 - DNA, 1143 bp, artificial
  Nucleic acid sequence of the biparatopic nanobody IGF-1269
caggtgcagcttgtacagtctgggggaggcttggtgcaggctggggggtctctgagactctcctgtgcagcctctgtaaggttcttcagtattaataccatgggctggtatcgccaggctccagggaagcagcgcgagttggtcgcagatattactagtagtggtagcacaaactatgcagactccgggaagggccgattcaccatctccagagacaacgccaagaacacggtgtatctgcagatgaacaggttgaaacctgaggacacagccgtctattactgccatgcggattacaaatacacaacccataacacggcctggggccagggtacccaggtcaccgtctcctcaggtgggggtggcagcggtggcggcggtagcgggggcggtggcagccaggtgcaattggtgcagtctgggggaggattggtgcaggctgggggctctctgagactctcctgtgcagcctctggacgcacctttagtagcttcgccatggcctggttccgccaggctccagggaaggagcgtgagtttgtagcagctattagctggagtggtagtacaggccatgcagactctgtgaagggccgattcaccatcaccagagacaacgccaagaacacggtgtttctgcaaatgaacagcctgaaacctgaggacacggccgtttattactgtgcactaggaaaggggagtagttactactacagtcctagtgggtatgactactggggccaggggacccaggtcaccgtctcctcaggtgggggtggcagcggtggcggcggtagccaggtgcagctgcaagaaagcggagggggcctggtccagccaggaggcagcctccggctaagttgcgaggccagcggcttcacattcagtagatttggcatgacatgggtcaggcaggccccaggtaaaggcgtggaatgggtaagcggcataagcagtctgggagacagcacactctacgccgattccgtgaaaggccgcttcaccatctctagagacaacgcaaaaaataccctgtaccttcagatgaattcactcaagcccgaagacacggccgtttattactgcacaatcggcgggtcactaaacccaggcggacaggggacacaagtaacggttagtagc

SEQ ID NO: 53 - DNA, 1185 bp, artificial
  Nucleic acid sequence of the biparatopic nanobody IGF-1270
caggtgcagcttgtacagtctgggggaggcttggtgcaggctggggggtctctgagactctcctgtgcagcctctgtaaggttcttcagtattaataccatgggctggtatcgccaggctccagggaagcagcgcgagttggtcgcagatattactagtagtggtagcacaaactatgcagactccgggaagggccgattcaccatctccagagacaacgccaagaacacggtgtatctgcagatgaacaggttgaaacctgaggacacagccgtctattactgccatgcggattacaaatacacaacccataacacggcctggggccagggtacccaggtcaccgtctcctcagaaccgaagatcccgcagccgcagccaaaacctcagccgcagccacagccgcaacctcaaccgaaaccgcaaccaaaaccggaacctcaggtgcaattggtgcagtctgggggaggattggtgcaggctgggggctctctgagactctcctgtgcagcctctggacgcacctttagtagcttcgccatggcctggttccgccaggctccagggaaggagcgtgagtttgtagcagctattagctggagtggtagtacaggccatgcagactctgtgaagggccgattcaccatcaccagagacaacgccaagaacacggtgtttctgcaaatgaacagcctgaaacctgaggacacggccgtttattactgtgcactaggaaaggggagtagttactactacagtcctagtgggtatgactactggggccaggggacccaggtcaccgtctcctcaggtgggggtggcagcggtggcggcggtagccaggtgcagctgcaagaaagcggagggggcctggtccagccaggaggcagcctccggctaagttgcgaggccagcggcttcacattcagtagatttggcatgacatgggtcaggcaggccccaggtaaaggcgtggaatgggtaagcggcataagcagtctgggagacagcacactctacgccgattccgtgaaaggccgcttcaccatctctagagacaacgcaaaaaataccctgtaccttcagatgaattcactcaagcccgaagacacggccgtttattactgcacaatcggcgggtcactaaacccaggcggacaggggacacaagtaacggttagtagc